European Patent Specification EP 3 378 947 B1, published January 24, 2024. Title: Use of ED-B protein in diagnosis of tissue hyperplasia. Applicant: Hefei Lifeon Pharmaceutical Co. Ltd. Application 15908514.1. The sequence listing filed with the application follows.

SEQUENCE LISTING (3 sequences)

SEQ ID NO: 1 - protein, 91 aa, Homo sapiens
EVPQLTDLSFVDITDSSIGLRWTPLNSSTIIGYRITVVAAGEGIPIFEDFVDSSVGYYTVTGLEPGIDYDISVITLINGGESAPTTLTQQT

SEQ ID NO: 2 - DNA, 273 bp, Homo sapiens
gaggtgccccaactcactgacctaagctttgttgatataaccgattcaagcatcggcctgaggtggaccccgctaaactcttccaccattattgggtaccgcatcacagtagttgcggcaggagaaggtatccctatttttgaagattttgtggactcctcagtaggatactacacagtcacagggctggagccgggcattgactatgatatcagcgttatcactctcattaatggcggcgagagtgcccctactacactgacacaacaaacg

SEQ ID NO: 3 - DNA, 900 bp, Artificial Sequence
  encoding 3 FN(7B8)
gctagcatggagaccgacaccctcctgctgtgggtgctgctgctctgggtgcccggctccaccggcgacggcccattgtctccaccaacaaacttgcatctggaggcaaaccctgacactggagtgctcacagtctcctgggagaggagcaccaccccagacattactggttatagaattaccacaacccctacaaacggccagcagggaaattctttggaagaagtggtccatgctgatcagagctcctgcacttttgataacctgagtcccggcctggagtacaatgtcagtgtttacactgtcaaggatgacaaggaaagtgtccctatctctgataccatcatcccagaggtgccccaactcactgacctaagctttgttgatataaccgattcaagcatcggcctgaggtggaccccgctaaactcttccaccattattgggtaccgcatcacagtagttgcggcaggagaaggtatccctatttttgaagattttgtggactcctcagtaggatactacacagtcacagggctggagccgggcattgactatgatatcagcgttatcactctcattaatggcggcgagagtgcccctactacactgacacaacaaacggctgttcctcctcccactgacctgcgattcaccaacattggtccagacaccatgcgtgtcacctgggctccacccccatccattgatttaaccaacttcctggtgcgttactcacctgtgaaaaatgaggaagatgttgcagagttgtcaatttctccttcagacaatgcagtggtcttaacaaatctcctgcctggtacagaatatgtagtgagtgtctccagtgtctacgaacaacatgagagcacacctcttagaggaagacagaaaacaggt